European Patent Specification EP 3 807 407 B1, published December 3, 2025. Title: Selection System For Evolving Proteases and Protease-Cleavage Sites. Applicant: Max-Planck-Gesellschaft zur Förderung der Wissenschaften e.V. The sequence listing filed with the application follows.

SEQUENCE LISTING (72 sequences)

SEQ ID NO: 1 - protein, 5 aa, Artificial
  DegronNER
FLFVQ

SEQ ID NO: 2 - protein, 10 aa, Artificial
  ssrA
AADENYALAA

SEQ ID NO: 3 - protein, 97 aa, Artificial
  Wt bdSUMO
MSAAGGEEDKKPAGGEGGGAHINLKVKGQDGNEVFFRIKRSTQLKKLMNAYCDRQSVDMTAIAFLFDGRRLRAEQTPDELEMEDGDEIDAMLHQTGG

SEQ ID NO: 4 - protein, 98 aa, Artificial
  scSUMO/Smt3p
MSDSEVNQEAKPEVKPEVKPETHINLKVSDGSSEIFFKIKKTTPLRRLMEAFAKRQGKEMDSLRFLYDGIRIQADQTPEDLDMEDNDIIEAHREQIGG

SEQ ID NO: 5 - protein, 93 aa, Artificial
  hsSUMO2
MADEKPKEGVKTENNDHINLKVAGQDGSVVQFKIKRHTPLSKLMKAYCERQGLSMRQIRFRFDGQPINETDTPAQLEMEDEDTIDVFQQQTGG

SEQ ID NO: 6 - protein, 234 aa, Artificial
  bdSENP1
PFVPLTDEDEDNVRHALGGRKRSETLSVHEASNIVITREILQCLNDKEWLNDEVINLYLELLKERELREPNKFLKCHFFNTFFYKKLINGGYDYKSVRRWTTKRKLGYNLIDCDKIFVPIHKDVHWCLAVINIKEKKFQYLDSLGYMDMKALRILAKYLVDEVKDKSGKQIDVHAWKQEGVQNLPLQENGWDCGMFMLKYIDFYSRDMELVFGQKHMSYFRRRTAKEILDLKAG

SEQ ID NO: 7 - protein, 219 aa, Artificial
  scUlp1
LVPELNEKDDDQVQKALASRENTQLMNRDNIEITVRDFKTLAPRRWLNDTIIEFFMKYIEKSTPNTVAFNSFFYTNLSERGYQGVRRWMKRKKTQIDKLDKIFTPINLNQSHWALGIIDLKKKTIGYVDSLSNGPNAMSFAILTDLQKYVMEESKHTIGEDFDLIHLDCPQQPNGYDCGIYVCMNTLYGSADAPLDFDYKDAIRMRRFIAHLILTDALK

SEQ ID NO: 8 - protein, 226 aa, Artificial
  hsSENP2
EFPEITEEMEKEIKNVFRNGNQDEVLSEAFRLTITRKDIQTLNHLNWLNDEIINFYMNMLMERSKEKGLPSVHAFNTFFFTKLKTAGYQAVKRWTKKVDVFSVDILLVPIHLGVHWCLAVVDFRKKNITYYDSMGGINNEACRILLQYLKQESIDKKRKEFDTNGWQLFSKKSQEIPQQMNGSDCGMFACKYADCITKDRPINFTQQHMPYFRKRMVWEILHRKLL

SEQ ID NO: 9 - protein, 24 aa, Artificial
  Wt bdSUMO; amino acids 56-79
SVDMTAIAFLFDGRRLRAEQTPDE

SEQ ID NO: 10 - protein, 24 aa, Artificial
  Mut1 bdSUMO
SVDMKAIAFLFKGRRLRAERTPDE

SEQ ID NO: 11 - protein, 24 aa, Artificial
  Mut2 bdSUMO
SVDMTAIAFLFKGRRLRAECTPDE

SEQ ID NO: 12 - protein, 24 aa, Artificial
  Mut3 bdSUMO
SVDMHAIAFLFKGRRLRAEKTPDE

SEQ ID NO: 13 - protein, 24 aa, Artificial
  Mut4 bdSUMO
SVDMRAIAFLFRGRRLRAEVTPDE

SEQ ID NO: 14 - protein, 24 aa, Artificial
  Mut5 bdSUMO
SVDMTAIAFLFKGRRLRAEFTPDE

SEQ ID NO: 15 - protein, 24 aa, Artificial
  Mut6 bdSUMO
SVDMHAIAFLFKGRRLRAEQTPDE

SEQ ID NO: 16 - protein, 24 aa, Artificial
  Mut7 bdSUMO
SVDMDAIAFLFRGRRLRAECTPDE

SEQ ID NO: 17 - protein, 24 aa, Artificial
  Mut8 bdSUMO
SVDMPAIAFLFKGRRLRAEWTPDE

SEQ ID NO: 18 - protein, 24 aa, Artificial
  Mut9 bdSUMO
SVDMAAIAFLFKGRRLRAEYTPDE

SEQ ID NO: 19 - protein, 24 aa, Artificial
  Mut10 bdSUMO
SVDMTAIAFLFKGRRLRAERTPDE

SEQ ID NO: 20 - protein, 24 aa, Artificial
  Mut11 bdSUMO
SVDMSAIAFLFKGRRLRAEWTPDE

SEQ ID NO: 21 - protein, 24 aa, Artificial
  Mut12 bdSUMO
SVDMSAIAFLFKGRRLRAEHTPDE

SEQ ID NO: 22 - protein, 24 aa, Artificial
  Mut13 bdSUMO
SVDMSAIAFLFKGRRLRAEATPDE

SEQ ID NO: 23 - protein, 24 aa, Artificial
  Mut14 bdSUMO
SVDMNAIAFLFKGRRLRAEWTPDE

SEQ ID NO: 24 - protein, 24 aa, Artificial
  Mut15 bdSUMO
SVDMNAIAFLFKGRRLRAEATPDE

SEQ ID NO: 25 - protein, 90 aa, Artificial
  Wt bdSENP1
GGRKRSETLSVHEASNIVITREILQCLNDKEWLNDEVINLYLELLKERELREPNKFLKCHFFNTFFYKKLINGGYDYKSVRRWTTKRKLG

SEQ ID NO: 26 - protein, 90 aa, Artificial
  MutA bdSENP1
GGRKPSETLSVHEASGIVITREILQCLNDKEWLNDEVINLYLELLKERELREPNKFLKCHFFNTFFYKKLINGGYDYKSVREWTTPRKLG

SEQ ID NO: 27 - protein, 90 aa, Artificial
  MutB bdSENP1
GGRKRSETLSVHEASSIVITREILQCLNDKEWLNDEVINLYLELLKERELREPNKFLKCHFFNTFFYKKLINGGYDYKSVREWTTKRKLG

SEQ ID NO: 28 - protein, 90 aa, Artificial
  MutC bdSENP1
GGRKSSETLSVHEASAIVITREILQCLNDKEWLNDEVINLYLELLKERELREPNKFLKCHFFNTFFYKKLINGGYDYKSVRGWTTVRKLG

SEQ ID NO: 29 - protein, 90 aa, Artificial
  MutD bdSENP1
GGRKPSETLSVHEASEIVITREILQCLNDKEWLNDEVINLYLELLKERELREPNKFLKCHFFNTFFYKKLINGGYDYKSVREWTTQRKLG

SEQ ID NO: 30 - protein, 90 aa, Artificial
  MutE bdSENP1
GGRKRSETLSVHEASGIVITREILQCLNDKEWLNDEVINLYLELLKERELREPNKFLKCHFFNTFFYKKLINGGYDYKSVRYWTTARKLG

SEQ ID NO: 31 - protein, 90 aa, Artificial
  MutF bdSENP1
GGRKPSETLSVHEASCIVITREILQCLNDKEWLNDEVINLYLELLKERELREPNKFLKCHFFNTFFYKKLINGGYDYKSVRLWTTRRKLG

SEQ ID NO: 32 - protein, 89 aa, Artificial
  MutG bdSENP1
GGRKSSETLSVHEASHIVITREILQCLNDKEWLNDEVINLYLELLKERELREPNKFLKCHFFNTFFYKKLINGGYDYKSVRRWTTVKLG

SEQ ID NO: 33 - protein, 89 aa, Artificial
  MutH bdSENP1
GGRKPSETLSVHEASAIVITREILQCLNDKEWLNDEVINLYLELLKERELREPNKFLKCHFFNTFFYKKLINGYDYKSVREWTTMRKLG

SEQ ID NO: 34 - protein, 90 aa, Artificial
  Muti bdSENP1
GGRKKSETLSVHEASHIVITREILQCLNDKEWLNDEVINLYLELLKERELREPNKFLKCHFFNTFFYKKLINGGYDYKSVREWTTRRKLG

SEQ ID NO: 35 - protein, 90 aa, Artificial
  MutJ bdSENP1
GGRKESETLSVHEASSIVITREILQCLNDKEWLNDEVINLYLELLKERELREPNKFLKCHFFNTFFYKKLINGGYDYKSVRSWTTTRKLG

SEQ ID NO: 36 - protein, 90 aa, Artificial
  MutK bdSENP1
GGRKVSETLSVHEASQIVITREILQCLNDKEWLNDEVINLYLELLKERELREPNKFLKCHFFNTFFYKKLINGGYDYKSVRVWTTGRKLG

SEQ ID NO: 37 - protein, 90 aa, Artificial
  MutL bdSENP1
GGRKLSETLSVHEASVIVITREILQCLNDKEWLNDEVINLYLELLKERELREPNKFLKCHFFNTFFYKKLINGGYDYKSVRPWTTARKLG

SEQ ID NO: 38 - protein, 90 aa, Artificial
  MutM bdSENP1
GGRKASETLSVHEASWIVITREILQCLNDKEWLNDEVINLYLELLKERELREPNKFLKCHFFNTFFYKKLINGGYDYKSVRRWTTERKLG

SEQ ID NO: 39 - protein, 90 aa, Artificial
  MutN bdSENP1
GGRKSSETLSVHEASPIVITREILQCLNDKEWLNDEVINLYLELLKERELREPNKFLKCHFFNTFFYKKLINGGYDYKSVRRWTTRRKLG

SEQ ID NO: 40 - protein, 90 aa, Artificial
  MutO bdSENP1
GGRKRSETLSVHEASRIVITREILQCLNDKEWLNDEVINLYLELLKERELREPNKFLKCHFFNTFFYKKLINGGYDYKSVRGWTTLRKLG

SEQ ID NO: 41 - protein, 97 aa, Artificial
  Mut1 bdSUMO residues 1-97
MSAAGGEEDKKPAGGEGGGAHINLKVKGQDGNEVFFRIKRSTQLKKLMNAYCDRQSVDMKAIAFLFKGRRLRAERTPDELEMEDGDEIDAMLHQTGG

SEQ ID NO: 42 - protein, 97 aa, Artificial
  Mut2 bdSUMO residues 1-97
MSAAGGEEDKKPAGGEGGGAHINLKVKGQDGNEVFFRIKRSTQLKKLMNAYCDRQSVDMTAIAFLFKGRRLRAECTPDELEMEDGDEIDAMLHQTGG

SEQ ID NO: 43 - protein, 97 aa, Artificial
  Mut3 bdSUMO residues 1-97
MSAAGGEEDKKPAGGEGGGAHINLKVKGQDGNEVFFRIKRSTQLKKLMNAYCDRQSVDMHAIAFLFKGRRLRAEKTPDELEMEDGDEIDAMLHQTGG

SEQ ID NO: 44 - protein, 97 aa, Artificial
  Mut4 bdSUMO residues 1-97
MSAAGGEEDKKPAGGEGGGAHINLKVKGQDGNEVFFRIKRSTQLKKLMNAYCDRQSVDMRAIAFLFRGRRLRAEVTPDELEMEDGDEIDAMLHQTGG

SEQ ID NO: 45 - protein, 97 aa, Artificial
  Mut5 bdSUMO residues 1-97
MSAAGGEEDKKPAGGEGGGAHINLKVKGQDGNEVFFRIKRSTQLKKLMNAYCDRQSVDMTAIAFLFKGRRLRAEFTPDELEMEDGDEIDAMLHQTGG

SEQ ID NO: 46 - protein, 97 aa, Artificial
  Mut6 bdSUMO residues 1-97
MSAAGGEEDKKPAGGEGGGAHINLKVKGQDGNEVFFRIKRSTQLKKLMNAYCDRQSVDMHAIAFLFKGRRLRAEQTPDELEMEDGDEIDAMLHQTGG

SEQ ID NO: 47 - protein, 97 aa, Artificial
  Mut7 bdSUMO residues 1-97
MSAAGGEEDKKPAGGEGGGAHINLKVKGQDGNEVFFRIKRSTQLKKLMNAYCDRQSVDMDAIAFLFRGRRLRAECTPDELEMEDGDEIDAMLHQTGG

SEQ ID NO: 48 - protein, 97 aa, Artificial
  Mut8 bdSUMO residues 1-97
MSAAGGEEDKKPAGGEGGGAHINLKVKGQDGNEVFFRIKRSTQLKKLMNAYCDRQSVDMPAIAFLFKGRRLRAEQTPDELEMEDGDEIDAMLHQTGG

SEQ ID NO: 49 - protein, 97 aa, Artificial
  Mut9 bdSUMO residues 1-97
MSAAGGEEDKKPAGGEGGGAHINLKVKGQDGNEVFFRIKRSTQLKKLMNAYCDRQSVDMAAIAFLFKGRRLRAEYTPDELEMEDGDEIDAMLHQTGG

SEQ ID NO: 50 - protein, 97 aa, Artificial
  Mut10 bdSUMO residues 1-97
MSAAGGEEDKKPAGGEGGGAHINLKVKGQDGNEVFFRIKRSTQLKKLMNAYCDRQSVDMTAIAFLFKGRRLRAERTPDELEMEDGDEIDAMLHQTGG

SEQ ID NO: 51 - protein, 97 aa, Artificial
  Mut11 bdSUMO residues 1-97
MSAAGGEEDKKPAGGEGGGAHINLKVKGQDGNEVFFRIKRSTQLKKLMNAYCDRQSVDMSAIAFLFKGRRLRAEWTPDELEMEDGDEIDAMLHQTGG

SEQ ID NO: 52 - protein, 97 aa, Artificial
  Mut12 bdSUMO residues 1-97
MSAAGGEEDKKPAGGEGGGAHINLKVKGQDGNEVFFRIKRSTQLKKLMNAYCDRQSVDMSAIAFLFKGRRLRAEHTPDELEMEDGDEIDAMLHQTGG

SEQ ID NO: 53 - protein, 97 aa, Artificial
  Mut13 bdSUMO residues 1-97
MSAAGGEEDKKPAGGEGGGAHINLKVKGQDGNEVFFRIKRSTQLKKLMNAYCDRQSVDMSAIAFLFKGRRLRAEATPDELEMEDGDEIDAMLHQTGG

SEQ ID NO: 54 - protein, 97 aa, Artificial
  Mut14 bdSUMO residues 1-97
MSAAGGEEDKKPAGGEGGGAHINLKVKGQDGNEVFFRIKRSTQLKKLMNAYCDRQSVDMNAIAFLFKGRRLRAEWTPDELEMEDGDEIDAMLHQTGG

SEQ ID NO: 55 - protein, 97 aa, Artificial
  Mut15 bdSUMO residues 1-97
MSAAGGEEDKKPAGGEGGGAHINLKVKGQDGNEVFFRIKRSTQLKKLMNAYCDRQSVDMNAIAFLFKGRRLRAEATPDELEMEDGDEIDAMLHQTGG

SEQ ID NO: 56 - protein, 234 aa, Artificial
  MutA bdSENP1 residues 248-481
PFVPLTDEDEDNVRHALGGRKPSETLSVHEASGIVITREILQCLNDKEWLNDEVINLYLELLKERELREPNKFLKCHFFNTFFYKKLINGGYDYKSVREWTTPRKLGYNLIDCDKIFVPIHKDVHWCLAVINIKEKKFQYLDSLGYMDMKALRILAKYLVDEVKDKSGKQIDVHAWKQEGVQNLPLQENGWDCGMFMLKYIDFYSRDMELVFGQKHMSYFRRRTAKEILDLKAG

SEQ ID NO: 57 - protein, 234 aa, Artificial
  MutB bdSENP1 residues 248-481
PFVPLTDEDEDNVRHALGGRKRSETLSVHEASSIVITREILQCLNDKEWLNDEVINLYLELLKERELREPNKFLKCHFFNTFFYKKLINGGYDYKSVREWTTKRKLGYNLIDCDKIFVPIHKDVHWCLAVINIKEKKFQYLDSLGYMDMKALRILAKYLVDEVKDKSGKQIDVHAWKQEGVQNLPLQENGWDCGMFMLKYIDFYSRDMELVFGQKHMSYFRRRTAKEILDLKAG

SEQ ID NO: 58 - protein, 234 aa, Artificial
  MutC bdSENP1 residues 248-481
PFVPLTDEDEDNVRHALGGRKSSETLSVHEASAIVITREILQCLNDKEWLNDEVINLYLELLKERELREPNKFLKCHFFNTFFYKKLINGGYDYKSVRGWTTVRKLGYNLIDCDKIFVPIHKDVHWCLAVINIKEKKFQYLDSLGYMDMKALRILAKYLVDEVKDKSGKQIDVHAWKQEGVQNLPLQENGWDCGMFMLKYIDFYSRDMELVFGQKHMSYFRRRTAKEILDLKAG

SEQ ID NO: 59 - protein, 234 aa, Artificial
  MutD bdSENP1 residues 248-481
PFVPLTDEDEDNVRHALGGRKPSETLSVHEASEIVITREILQCLNDKEWLNDEVINLYLELLKERELREPNKFLKCHFFNTFFYKKLINGGYDYKSVREWTTQRKLGYNLIDCDKIFVPIHKDVHWCLAVINIKEKKFQYLDSLGYMDMKALRILAKYLVDEVKDKSGKQIDVHAWKQEGVQNLPLQENGWDCGMFMLKYIDFYSRDMELVFGQKHMSYFRRRTAKEILDLKAG

SEQ ID NO: 60 - protein, 234 aa, Artificial
  MutE bdSENP1 residues 248-481
PFVPLTDEDEDNVRHALGGRKRSETLSVHEASGIVITREILQCLNDKEWLNDEVINLYLELLKERELREPNKFLKCHFFNTFFYKKLINGGYDYKSVRYWTTARKLGYNLIDCDKIFVPIHKDVHWCLAVINIKEKKFQYLDSLGYMDMKALRILAKYLVDEVKDKSGKQIDVHAWKQEGVQNLPLQENGWDCGMFMLKYIDFYSRDMELVFGQKHMSYFRRRTAKEILDLKAG

SEQ ID NO: 61 - protein, 234 aa, Artificial
  MutF bdSENP1 residues 248-481
PFVPLTDEDEDNVRHALGGRKPSETLSVHEASCIVITREILQCLNDKEWLNDEVINLYLELLKERELREPNKFLKCHFFNTFFYKKLINGGYDYKSVRLWTTRRKLGYNLIDCDKIFVPIHKDVHWCLAVINIKEKKFQYLDSLGYMDMKALRILAKYLVDEVKDKSGKQIDVHAWKQEGVQNLPLQENGWDCGMFMLKYIDFYSRDMELVFGQKHMSYFRRRTAKEILDLKAG

SEQ ID NO: 62 - protein, 233 aa, Artificial
  MutG bdSENP1 residues 248-481
PFVPLTDEDEDNVRHALGGRKSSETLSVHEASHIVITREILQCLNDKEWLNDEVINLYLELLKERELREPNKFLKCHFFNTFFYKKLINGGYDYKSVRRWTTVKLGYNLIDCDKIFVPIHKDVHWCLAVINIKEKKFQYLDSLGYMDMKALRILAKYLVDEVKDKSGKQIDVHAWKQEGVQNLPLQENGWDCGMFMLKYIDFYSRDMELVFGQKHMSYFRRRTAKEILDLKAG

SEQ ID NO: 63 - protein, 233 aa, Artificial
  MutH bdSENP1 residues 248-481
PFVPLTDEDEDNVRHALGGRKPSETLSVHEASAIVITREILQCLNDKEWLNDEVINLYLELLKERELREPNKFLKCHFFNTFFYKKLINGYDYKSVREWTTMRKLGYNLIDCDKIFVPIHKDVHWCLAVINIKEKKFQYLDSLGYMDMKALRILAKYLVDEVKDKSGKQIDVHAWKQEGVQNLPLQENGWDCGMFMLKYIDFYSRDMELVFGQKHMSYFRRRTAKEILDLKAG

SEQ ID NO: 64 - protein, 234 aa, Artificial
  Muti bdSENP1 residues 248-481
PFVPLTDEDEDNVRHALGGRKKSETLSVHEASHIVITREILQCLNDKEWLNDEVINLYLELLKERELREPNKFLKCHFFNTFFYKKLINGGYDYKSVREWTTRRKLGYNLIDCDKIFVPIHKDVHWCLAVINIKEKKFQYLDSLGYMDMKALRILAKYLVDEVKDKSGKQIDVHAWKQEGVQNLPLQENGWDCGMFMLKYIDFYSRDMELVFGQKHMSYFRRRTAKEILDLKAG

SEQ ID NO: 65 - protein, 234 aa, Artificial
  MutJ bdSENP1 residues 248-481
PFVPLTDEDEDNVRHALGGRKESETLSVHEASSIVITREILQCLNDKEWLNDEVINLYLELLKERELREPNKFLKCHFFNTFFYKKLINGGYDYKSVRSWTTTRKLGYNLIDCDKIFVPIHKDVHWCLAVINIKEKKFQYLDSLGYMDMKALRILAKYLVDEVKDKSGKQIDVHAWKQEGVQNLPLQENGWDCGMFMLKYIDFYSRDMELVFGQKHMSYFRRRTAKEILDLKAG

SEQ ID NO: 66 - protein, 234 aa, Artificial
  MutK bdSENP1 residues 248-481
PFVPLTDEDEDNVRHALGGRKVSETLSVHEASQIVITREILQCLNDKEWLNDEVINLYLELLKERELREPNKFLKCHFFNTFFYKKLINGGYDYKSVRVWTTGRKLGYNLIDCDKIFVPIHKDVHWCLAVINIKEKKFQYLDSLGYMDMKALRILAKYLVDEVKDKSGKQIDVHAWKQEGVQNLPLQENGWDCGMFMLKYIDFYSRDMELVFGQKHMSYFRRRTAKEILDLKAG

SEQ ID NO: 67 - protein, 234 aa, Artificial
  MutL bdSENP1 residues 248-481
PFVPLTDEDEDNVRHALGGRKLSETLSVHEASVIVITREILQCLNDKEWLNDEVINLYLELLKERELREPNKFLKCHFFNTFFYKKLINGGYDYKSVRPWTTARKLGYNLIDCDKIFVPIHKDVHWCLAVINIKEKKFQYLDSLGYMDMKALRILAKYLVDEVKDKSGKQIDVHAWKQEGVQNLPLQENGWDCGMFMLKYIDFYSRDMELVFGQKHMSYFRRRTAKEILDLKAG

SEQ ID NO: 68 - protein, 234 aa, Artificial
  MutM bdSENP1 residues 248-481
PFVPLTDEDEDNVRHALGGRKASETLSVHEASWIVITREILQCLNDKEWLNDEVINLYLELLKERELREPNKFLKCHFFNTFFYKKLINGGYDYKSVRRWTTERKLGYNLIDCDKIFVPIHKDVHWCLAVINIKEKKFQYLDSLGYMDMKALRILAKYLVDEVKDKSGKQIDVHAWKQEGVQNLPLQENGWDCGMFMLKYIDFYSRDMELVFGQKHMSYFRRRTAKEILDLKAG

SEQ ID NO: 69 - protein, 234 aa, Artificial
  MutN bdSENP1 residues 248-481
PFVPLTDEDEDNVRHALGGRKSSETLSVHEASPIVITREILQCLNDKEWLNDEVINLYLELLKERELREPNKFLKCHFFNTFFYKKLINGGYDYKSVRRWTTRRKLGYNLIDCDKIFVPIHKDVHWCLAVINIKEKKFQYLDSLGYMDMKALRILAKYLVDEVKDKSGKQIDVHAWKQEGVQNLPLQENGWDCGMFMLKYIDFYSRDMELVFGQKHMSYFRRRTAKEILDLKAG

SEQ ID NO: 70 - protein, 234 aa, Artificial
  MutO bdSENP1 residues 248-481
PFVPLTDEDEDNVRHALGGRKRSETLSVHEASRIVITREILQCLNDKEWLNDEVINLYLELLKERELREPNKFLKCHFFNTFFYKKLINGGYDYKSVRGWTTLRKLGYNLIDCDKIFVPIHKDVHWCLAVINIKEKKFQYLDSLGYMDMKALRILAKYLVDEVKDKSGKQIDVHAWKQEGVQNLPLQENGWDCGMFMLKYIDFYSRDMELVFGQKHMSYFRRRTAKEILDLKAG

SEQ ID NO: 71 - protein, 373 aa, Artificial
  MBP fusion
AGTGTSKTEEGKLVIWINGDKGYNGLAEVGKKFEKDTGIKVTVEHPDKLEEKFPQVAATGDGPDIIFWAHDRFGGYAQSGLLAEITPDKAFQDKLYPFTWDAVRYNGKLIAYPIAVEALSLIYNKDLLPNPPKTWEEIPALDKELKAKGKSALMFNLQEPYFTWPLIAADGGYAFKYENGKYDIKDVGVDNAGAKAGLTFLVDLIKNKHMNADTDYSIAEAAFNKGETAMTINGPWAWSNIDTSKVNYGVTVLPTFKGQPSKPFVGVLSAGINAASPNKELAKEFLENYLLTDEGLEAVNKDKPLGAVALKSYEEELAKDPRIAATMENAQKGEIMPNIPQMSAFWYAVRTAVINAASGRQTVDEALKDAQTN

SEQ ID NO: 72 - RNA, 17 nt, Artificial
  RBS
aaaacaaguuauccaug